European Patent Specification EP 4 090 352 B1, published June 17, 2026. Title: ANIMAL MODELS OF LIPID METABOLISM AND METHODS OF TREATING HYPERLIPIDEMIA OR HYPERLIPIDEMIA-RELATED DISEASES. Applicant: Academia Sinica. The sequence listing filed with the application follows.

SEQUENCE LISTING (20 sequences)

SEQ ID NO: 1 - protein, 152 aa, Artificial Sequence
  synthesized_WT PRAP1_isoform CRA a
MKRFLLATCLVAALLWEAGAAPAHQVPVKTKGKHVFPEQETEKVGRVWDTRALEPLEKDNQLGPLLPEPKQKPAAAEEKRPDAMTWVETEDILSHLRSPLQGPELDLDSIDHPMSDDVQDEEVPQSRPILYRQVLQGPEEDLDHLAHSMEDS

SEQ ID NO: 2 - protein, 152 aa, Artificial Sequence
  synthesized_Mouse E88V mutant PRAP1
MKRFLLATCLVAALLWEAGAAPAHQVPVKTKGKHVFPEQETEKVGRVWDTRALEPLEKDNQLGPLLPEPKQKPAAAEEKRPDAMTWVVTEDILSHLRSPLQGPELDLDSIDHPMSDDVQDEEVPQSRPILYRQVLQGPEEDLDHLAHSMEDS

SEQ ID NO: 3 - protein, 149 aa, Artificial Sequence
  synthesized_WT PRAP1_isoform CRA b
MKRFLLATCLVAALLWEAGAAPAHQVPVKTKGKHVFPEQETEKVWDTRALEPLEKDNQLGPLLPEPKQKPAAAEEKRPDAMTWVETEDILSHLRSPLQGPELDLDSIDHPMSDDVQDEEVPQSRPILYRQVLQGPEEDLDHLAHSMEDS

SEQ ID NO: 4 - protein, 149 aa, Artificial Sequence
  synthesized_Mouse E85V mutant PRAP1
MKRFLLATCLVAALLWEAGAAPAHQVPVKTKGKHVFPEQETEKVWDTRALEPLEKDNQLGPLLPEPKQKPAAAEEKRPDAMTWVVTEDILSHLRSPLQGPELDLDSIDHPMSDDVQDEEVPQSRPILYRQVLQGPEEDLDHLAHSMEDS

SEQ ID NO: 5 - protein, 151 aa, Artificial Sequence
  synthesized_WT PRAP1_variant 1
MRRLLLVTSLVVVLLWEAGAVPAPKVPIKMQVKHWPSEQDPEKAWGARVVEPPEKDDQLVVLFPVQKPKLLTTEEKPRGQGRGPILPGTKAWMETEDTLGHVLSPEPDHDSLYHPPPEEDQGEERPRLWVMPNHQVLLGPEEDQDHIYHPQ

SEQ ID NO: 6 - protein, 151 aa, Artificial Sequence
  synthesized_Human E94V mutant PRAP1
MRRLLLVTSLVVVLLWEAGAVPAPKVPIKMQVKHWPSEQDPEKAWGARVVEPPEKDDQLVVLFPVQKPKLLTTEEKPRGQGRGPILPGTKAWMVTEDTLGHVLSPEPDHDSLYHPPPEEDQGEERPRLWVMPNHQVLLGPEEDQDHIYHPQ

SEQ ID NO: 7 - protein, 142 aa, Artificial Sequence
  synthesized_WT PRAP1_variant 2
MRRLLLVTSLVVVLLWEAGAVPAPKVPIKMQVKHWPSEQDPEKAWGARVVEPPEKDDQLVVLFPVQKPKLLTTEEKPRGTKAWMETEDTLGHVLSPEPDHDSLYHPPPEEDQGEERPRLWVMPNHQVLLGPEEDQDHIYHPQ

SEQ ID NO: 8 - protein, 142 aa, Artificial Sequence
  synthesized_Human E85V mutant PRAP1
MRRLLLVTSLVVVLLWEAGAVPAPKVPIKMQVKHWPSEQDPEKAWGARVVEPPEKDDQLVVLFPVQKPKLLTTEEKPRGTKAWMVTEDTLGHVLSPEPDHDSLYHPPPEEDQGEERPRLWVMPNHQVLLGPEEDQDHIYHPQ

SEQ ID NO: 9 - protein, 9 aa, Artificial Sequence
  synthesized_difference sequence between variants 1 and 2
QGRGPILPG

SEQ ID NO: 10 - DNA, 23 bp, Artificial Sequence
  synthesized_p1 primer
tccagcacaccaggtatgcaagg

SEQ ID NO: 11 - DNA, 23 bp, Artificial Sequence
  synthesized_p3 primer
agggtcctcaagggcaagggagt

SEQ ID NO: 12 - DNA, 22 bp, Artificial Sequence
  synthesized_p2 primer
tcgatagcttggctgcaggtcg

SEQ ID NO: 13 - DNA, 129 bp, Artificial Sequence
  synthesized_mutant DNA oligo
gtgggaaggatcttgtgagggaggctatatctacgtctccttctccacagatgccatgacatgggtagtgactgaggatatcctgagccatcttcgcagtcctcttcagggtccagaactggatcttga

SEQ ID NO: 14 - DNA, 20 bp, Artificial Sequence
  synthesized_sgRNA
gatatcctcagtctccaccc

SEQ ID NO: 15 - DNA, 20 bp, Artificial Sequence
  synthesized_PRAP1-I3-F
tacctactcccttgcccttg

SEQ ID NO: 16 - DNA, 20 bp, Artificial Sequence
  synthesized_PRAP1-reverse
cagtctccacccaggtcatg

SEQ ID NO: 17 - DNA, 20 bp, Artificial Sequence
  synthesized_E85V-reverse
cagtcactacccatgtcatg

SEQ ID NO: 18 - DNA, 6636 bp, Artificial Sequence
  synthesized_LacZ-Neo cassette
gtcgacctgcagccaagctatcgaattccgcccctctccctcccccccccctaacgttactggccgaagccgcttggaataaggccggtgagcgtttgtctatatgttattttccaccatattgccgtcttttggcaatgtgagggcccgaaacctggccctgtcttcttgacgacgattcctaggggtctttcccctctcgccaaaggaatgcaaggtctgttgaatgtcgtgaaggaagcagttcctctggaagcttcttgaagacaacaacgtctgtagcgaccctttgcaggcagcggaaccccccacctggcgacatggatagttgtggaaagagtcaaatggctctcctcaagcgtattcaacaaggggctgaaggatgcccagaaggtaccccattgtatgggatctgatctggggcctcggtgcacatgctttacatgtgtttagtcgaggttaaaaaacgtctaggccccccgaaccacggggacgtggttttggtttgaaaaacacgatgataatatggccacaaccatggaacagggggatgagcttaccatggccaagatccctcctaagaagaagcgcaaagtcgaggatcccgtcgttttacaacgtcgtgactgggaaaaccctggcgttacccaacttaatcgccttgcagcacatccccctttcgccagctggcgtaatagcgaagaggcccgcaccgatcgcccttcccaacagttgcgcagcctgaatggcgaatggcgctttgcctggtttccggcaccagaagcggtgccggaaagctggctggagtgcgatcttcctgaggccgatactgtcgtcgtcccctcaaactggcagatgcacggttacgatgcgcccatctacaccaacgtaacctatcccattacggtcaatccgccgtttgttcccacggagaatccgacgggttgttactcgctcacatttaatgttgatgaaagctggctacaggaaggccagacgcgaattatttttgatggcgttaactcggcgtttcatctgtggtgcaacgggcgctgggtcggttacggccaggacagtcgtttgccgtctgaatttgacctgagcgcatttttacgcgccggagaaaaccgcctcgcggtgatggtgctgcgttggagtgacggcagttatctggaagatcaggatatgtggcggatgagcggcattttccgtgacgtctcgttgctgcataaaccgactacacaaatcagcgatttccatgttgccactcgctttaatgatgatttcagccgcgctgtactggaggctgaagttcagatgtgcggcgagttgcgtgactacctacgggtaacagtttctttatggcagggtgaaacgcaggtcgccagcggcaccgcgcctttcggcggtgaaattatcgatgagcgtggtggttatgccgatcgcgtcacactacgtctgaacgtcgaaaacccgaaactgtggagcgccgaaatcccgaatctctatcgtgcggtggttgaactgcacaccgccgacggcacgctgattgaagcagaagcctgcgatgtcggtttccgcgaggtgcggattgaaaatggtctgctgctgctgaacggcaagccgttgctgattcgaggcgttaaccgtcacgagcatcatcctctgcatggtcaggtcatggatgagcagacgatggtgcaggatatcctgctgatgaagcagaacaactttaacgccgtgcgctgttcgcattatccgaaccatccgctgtggtacacgctgtgcgaccgctacggcctgtatgtggtggatgaagccaatattgaaacccacggcatggtgccaatgaatcgtctgaccgatgatccgcgctggctaccggcgatgagcgaacgcgtaacgcgaatggtgcagcgcgatcgtaatcacccgagtgtgatcatctggtcgctggggaatgaatcaggccacggcgctaatcacgacgcgctgtatcgctggatcaaatctgtcgatccttcccgcccggtgcagtatgaaggcggcggagccgacaccacggccaccgatattatttgcccgatgtacgcgcgcgtggatgaagaccagcccttcccggctgtgccgaaatggtccatcaaaaaatggctttcgctacctggagagacgcgcccgctgatcctttgcgaatacgcccacgcgatgggtaacagtcttggcggtttcgctaaatactggcaggcgtttcgtcagtatccccgtttacagggcggcttcgtctgggactgggtggatcagtcgctgattaaatatgatgaaaacggcaacccgtggtcggcttacggcggtgattttggcgatacgccgaacgatcgccagttctgtatgaacggtctggtctttgccgaccgcacgccgcatccagcgctgacggaagcaaaacaccagcagcagtttttccagttccgtttatccgggcaaaccatcgaagtgaccagcgaatacctgttccgtcatagcgataacgagctcctgcactggatggtggcgctggatggtaagccgctggcaagcggtgaagtgcctctggatgtcgctccacaaggtaaacagttgattgaactgcctgaactaccgcagccggagagcgccgggcaactctggctcacagtacgcgtagtgcaaccgaacgcgaccgcatggtcagaagccgggcacatcagcgcctggcagcagtggcgtctggcggaaaacctcagtgtgacgctccccgccgcgtcccacgccatcccgcatctgaccaccagcgaaatggatttttgcatcgagctgggtaataagcgttggcaatttaaccgccagtcaggctttctttcacagatgtggattggcgataaaaaacaactgctgacgccgctgcgcgatcagttcacccgtgcaccgctggataacgacattggcgtaagtgaagcgacccgcattgaccctaacgcctgggtcgaacgctggaaggcggcgggccattaccaggccgaagcagcgttgttgcagtgcacggcagatacacttgctgatgcggtgctgattacgaccgctcacgcgtggcagcatcaggggaaaaccttatttatcagccggaaaacctaccggattgatggtagtggtcaaatggcgattaccgttgatgttgaagtggcgagcgatacaccgcatccggcgcggattggcctgaactgccagctggcgcaggtagcagagcgggtaaactggctcggattagggccgcaagaaaactatcccgaccgccttactgccgcctgttttgaccgctgggatctgccattgtcagacatgtataccccgtacgtcttcccgagcgaaaacggtctgcgctgcgggacgcgcgaattgaattatggcccacaccagtggcgcggcgacttccagttcaacatcagccgctacagtcaacagcaactgatggaaaccagccatcgccatctgctgcacgcggaagaaggcacatggctgaatatcgacggtttccatatggggattggtggcgacgactcctggagcccgtcagtatcggcggaattccagctgagcgccggtcgctaccattaccagttggtctggtgtcaaaaatattgtgaaggaaccttacttctgtggtgtgacataattggacaaactacctacagagatttaaagctctaaggtaaatataaaatttttaagtgtataatgtgttaaactactgattctaattgtttgtgtattttagattccaacctatggaactgatgaatgggagcagtggtggaatgcctttaatgaggaaaacctgttttgctcagaagaaatgccatctagtgatgatgaggctactgctgactctcaacattctactcctccaaaaaagaagagaaaggtagaagaccccaaggactttccttcagaattgctaagttttttgagtcatgctgtgtttagtaatagaactcttgcttgctttgctatttacaccacaaaggaaaaagctgcactgctatacaagaaaattatggaaaaatattctgtaacctttataagtaggcataacagttataatcataacatactgttttttcttactccacacaggcatagagtgtctgctattaataactatgctcaaaaattgtgtacctttagctttttaatttgtaaaggggttaataaggaatatttgatgtatagtgccttgactagagatcataatcagccataccacatttgtagaggttttacttgctttaaaaaacctcccacacctccccctgaacctgaaacataaaatgaatgcaattgttgttgttaacttgtttattgcagcttataatggttacaaataaagcaatagcatcacaaatttcacaaataaagcatttttttcactgcattctagttgtggtttgtccaaactcatcaatgtatcttatcatgtctggatccccaggaagctcctctgtgtcctcataaaccctaacctcctctacttgagaggacattccaatcataggctgcccatccaccctctgtgtcctcctgttaattaggtcacttaacaaaaaggaaattgggtaggggtttttcacagaccgctttctaagggtaattttaaaatatctgggaagtcccttccactgctgtgttccagaagtgttggtaaacagcccacaaatgtcaacagcagaaacatacaagctgtcagctttgcacaagggcccggtacccatcgaattcctgcagcccaattccgatcatattcaataacccttaatataacttcgtataatgtatgctatacgaagttattaggtctgaagaggagtttacgtccagccaagctagcttggctgcaggtcgtcgaattctaccgggtaggggaggcgcttttcccaaggcagtctggagcatgcgctttagcagccccgctgggcacttggcgctacacaagtggcctctggcctcgcacacattccacatccaccggtaggcgccaaccggctccgttctttggtggccccttcgcgccaccttctactcctcccctagtcaggaagttcccccccgccccgcagctcgcgtcgtgcaggacgtgacaaatggaagtagcacgtctcactagtctcgtgcagatggacagcaccgctgagcaatggaagcgggtaggcctttggggcagcggccaatagcagctttgctccttcgctttctgggctcagaggctgggaaggggtgggtccgggggcgggctcaggggcgggctcaggggcggggcgggcgcccgaaggtcctccggaggcccggcattctgcacgcttcaaaagcgcacgtctgccgcgctgttctcctcttcctcatctccgggcctttcgacctgcagccaatatgggatcggccattgaacaagatggattgcacgcaggttctccggccgcttgggtggagaggctattcggctatgactgggcacaacagacaatcggctgctctgatgccgccgtgttccggctgtcagcgcaggggcgcccggttctttttgtcaagaccgacctgtccggtgccctgaatgaactgcaggacgaggcagcgcggctatcgtggctggccacgacgggcgttccttgcgcagctgtgctcgacgttgtcactgaagcgggaagggactggctgctattgggcgaagtgccggggcaggatctcctgtcatctcaccttgctcctgccgagaaagtatccatcatggctgatgcaatgcggcggctgcatacgcttgatccggctacctgcccattcgaccaccaagcgaaacatcgcatcgagcgagcacgtactcggatggaagccggtcttgtcgatcaggatgatctggacgaagagcatcaggggctcgcgccagccgaactgttcgccaggctcaaggcgcgcatgcccgacggcgatgatctcgtcgtgacccatggcgatgcctgcttgccgaatatcatggtggaaaatggccgcttttctggattcatcgactgtggccggctgggtgtggcggaccgctatcaggacatagcgttggctacccgtgatattgctgaagagcttggcggcgaatgggctgaccgcttcctcgtgctttacggtatcgccgctcccgattcgcagcgcatcgccttctatcgccttcttgacgagttcttctgaggggatcaattctctagagctcgctgatcagcctcgactgtgccttctagttgccagccatctgttgtttgcccctcccccgtgccttccttgaccctggaaggtgccactcccactgtcctttcctaataaaatgaggaaattgcatcgcattgtctgagtaggtgtcattctattctggggggtggggtggggcaggacagcaagggggaggattgggaagacaatagcaggcatgctggggatgcggtgggctctatggcttctgaggcggaaagaaccagctggggctcgactagagcttgcggaacccttaatataacttcgtataatgtatgctatacgaagttattaggtccctcgaggggatccactagttctagagcggccggg

SEQ ID NO: 19 - DNA, 6689 bp, Artificial Sequence
  synthesized_E3-LacZ-neo-E3
gtccctgtcaagaccaaagggtcgacctgcagccaagctatcgaattccgcccctctccctcccccccccctaacgttactggccgaagccgcttggaataaggccggtgagcgtttgtctatatgttattttccaccatattgccgtcttttggcaatgtgagggcccgaaacctggccctgtcttcttgacgacgattcctaggggtctttcccctctcgccaaaggaatgcaaggtctgttgaatgtcgtgaaggaagcagttcctctggaagcttcttgaagacaacaacgtctgtagcgaccctttgcaggcagcggaaccccccacctggcgacatggatagttgtggaaagagtcaaatggctctcctcaagcgtattcaacaaggggctgaaggatgcccagaaggtaccccattgtatgggatctgatctggggcctcggtgcacatgctttacatgtgtttagtcgaggttaaaaaacgtctaggccccccgaaccacggggacgtggttttggtttgaaaaacacgatgataatatggccacaaccatggaacagggggatgagcttaccatggccaagatccctcctaagaagaagcgcaaagtcgaggatcccgtcgttttacaacgtcgtgactgggaaaaccctggcgttacccaacttaatcgccttgcagcacatccccctttcgccagctggcgtaatagcgaagaggcccgcaccgatcgcccttcccaacagttgcgcagcctgaatggcgaatggcgctttgcctggtttccggcaccagaagcggtgccggaaagctggctggagtgcgatcttcctgaggccgatactgtcgtcgtcccctcaaactggcagatgcacggttacgatgcgcccatctacaccaacgtaacctatcccattacggtcaatccgccgtttgttcccacggagaatccgacgggttgttactcgctcacatttaatgttgatgaaagctggctacaggaaggccagacgcgaattatttttgatggcgttaactcggcgtttcatctgtggtgcaacgggcgctgggtcggttacggccaggacagtcgtttgccgtctgaatttgacctgagcgcatttttacgcgccggagaaaaccgcctcgcggtgatggtgctgcgttggagtgacggcagttatctggaagatcaggatatgtggcggatgagcggcattttccgtgacgtctcgttgctgcataaaccgactacacaaatcagcgatttccatgttgccactcgctttaatgatgatttcagccgcgctgtactggaggctgaagttcagatgtgcggcgagttgcgtgactacctacgggtaacagtttctttatggcagggtgaaacgcaggtcgccagcggcaccgcgcctttcggcggtgaaattatcgatgagcgtggtggttatgccgatcgcgtcacactacgtctgaacgtcgaaaacccgaaactgtggagcgccgaaatcccgaatctctatcgtgcggtggttgaactgcacaccgccgacggcacgctgattgaagcagaagcctgcgatgtcggtttccgcgaggtgcggattgaaaatggtctgctgctgctgaacggcaagccgttgctgattcgaggcgttaaccgtcacgagcatcatcctctgcatggtcaggtcatggatgagcagacgatggtgcaggatatcctgctgatgaagcagaacaactttaacgccgtgcgctgttcgcattatccgaaccatccgctgtggtacacgctgtgcgaccgctacggcctgtatgtggtggatgaagccaatattgaaacccacggcatggtgccaatgaatcgtctgaccgatgatccgcgctggctaccggcgatgagcgaacgcgtaacgcgaatggtgcagcgcgatcgtaatcacccgagtgtgatcatctggtcgctggggaatgaatcaggccacggcgctaatcacgacgcgctgtatcgctggatcaaatctgtcgatccttcccgcccggtgcagtatgaaggcggcggagccgacaccacggccaccgatattatttgcccgatgtacgcgcgcgtggatgaagaccagcccttcccggctgtgccgaaatggtccatcaaaaaatggctttcgctacctggagagacgcgcccgctgatcctttgcgaatacgcccacgcgatgggtaacagtcttggcggtttcgctaaatactggcaggcgtttcgtcagtatccccgtttacagggcggcttcgtctgggactgggtggatcagtcgctgattaaatatgatgaaaacggcaacccgtggtcggcttacggcggtgattttggcgatacgccgaacgatcgccagttctgtatgaacggtctggtctttgccgaccgcacgccgcatccagcgctgacggaagcaaaacaccagcagcagtttttccagttccgtttatccgggcaaaccatcgaagtgaccagcgaatacctgttccgtcatagcgataacgagctcctgcactggatggtggcgctggatggtaagccgctggcaagcggtgaagtgcctctggatgtcgctccacaaggtaaacagttgattgaactgcctgaactaccgcagccggagagcgccgggcaactctggctcacagtacgcgtagtgcaaccgaacgcgaccgcatggtcagaagccgggcacatcagcgcctggcagcagtggcgtctggcggaaaacctcagtgtgacgctccccgccgcgtcccacgccatcccgcatctgaccaccagcgaaatggatttttgcatcgagctgggtaataagcgttggcaatttaaccgccagtcaggctttctttcacagatgtggattggcgataaaaaacaactgctgacgccgctgcgcgatcagttcacccgtgcaccgctggataacgacattggcgtaagtgaagcgacccgcattgaccctaacgcctgggtcgaacgctggaaggcggcgggccattaccaggccgaagcagcgttgttgcagtgcacggcagatacacttgctgatgcggtgctgattacgaccgctcacgcgtggcagcatcaggggaaaaccttatttatcagccggaaaacctaccggattgatggtagtggtcaaatggcgattaccgttgatgttgaagtggcgagcgatacaccgcatccggcgcggattggcctgaactgccagctggcgcaggtagcagagcgggtaaactggctcggattagggccgcaagaaaactatcccgaccgccttactgccgcctgttttgaccgctgggatctgccattgtcagacatgtataccccgtacgtcttcccgagcgaaaacggtctgcgctgcgggacgcgcgaattgaattatggcccacaccagtggcgcggcgacttccagttcaacatcagccgctacagtcaacagcaactgatggaaaccagccatcgccatctgctgcacgcggaagaaggcacatggctgaatatcgacggtttccatatggggattggtggcgacgactcctggagcccgtcagtatcggcggaattccagctgagcgccggtcgctaccattaccagttggtctggtgtcaaaaatattgtgaaggaaccttacttctgtggtgtgacataattggacaaactacctacagagatttaaagctctaaggtaaatataaaatttttaagtgtataatgtgttaaactactgattctaattgtttgtgtattttagattccaacctatggaactgatgaatgggagcagtggtggaatgcctttaatgaggaaaacctgttttgctcagaagaaatgccatctagtgatgatgaggctactgctgactctcaacattctactcctccaaaaaagaagagaaaggtagaagaccccaaggactttccttcagaattgctaagttttttgagtcatgctgtgtttagtaatagaactcttgcttgctttgctatttacaccacaaaggaaaaagctgcactgctatacaagaaaattatggaaaaatattctgtaacctttataagtaggcataacagttataatcataacatactgttttttcttactccacacaggcatagagtgtctgctattaataactatgctcaaaaattgtgtacctttagctttttaatttgtaaaggggttaataaggaatatttgatgtatagtgccttgactagagatcataatcagccataccacatttgtagaggttttacttgctttaaaaaacctcccacacctccccctgaacctgaaacataaaatgaatgcaattgttgttgttaacttgtttattgcagcttataatggttacaaataaagcaatagcatcacaaatttcacaaataaagcatttttttcactgcattctagttgtggtttgtccaaactcatcaatgtatcttatcatgtctggatccccaggaagctcctctgtgtcctcataaaccctaacctcctctacttgagaggacattccaatcataggctgcccatccaccctctgtgtcctcctgttaattaggtcacttaacaaaaaggaaattgggtaggggtttttcacagaccgctttctaagggtaattttaaaatatctgggaagtcccttccactgctgtgttccagaagtgttggtaaacagcccacaaatgtcaacagcagaaacatacaagctgtcagctttgcacaagggcccggtacccatcgaattcctgcagcccaattccgatcatattcaataacccttaatataacttcgtataatgtatgctatacgaagttattaggtctgaagaggagtttacgtccagccaagctagcttggctgcaggtcgtcgaattctaccgggtaggggaggcgcttttcccaaggcagtctggagcatgcgctttagcagccccgctgggcacttggcgctacacaagtggcctctggcctcgcacacattccacatccaccggtaggcgccaaccggctccgttctttggtggccccttcgcgccaccttctactcctcccctagtcaggaagttcccccccgccccgcagctcgcgtcgtgcaggacgtgacaaatggaagtagcacgtctcactagtctcgtgcagatggacagcaccgctgagcaatggaagcgggtaggcctttggggcagcggccaatagcagctttgctccttcgctttctgggctcagaggctgggaaggggtgggtccgggggcgggctcaggggcgggctcaggggcggggcgggcgcccgaaggtcctccggaggcccggcattctgcacgcttcaaaagcgcacgtctgccgcgctgttctcctcttcctcatctccgggcctttcgacctgcagccaatatgggatcggccattgaacaagatggattgcacgcaggttctccggccgcttgggtggagaggctattcggctatgactgggcacaacagacaatcggctgctctgatgccgccgtgttccggctgtcagcgcaggggcgcccggttctttttgtcaagaccgacctgtccggtgccctgaatgaactgcaggacgaggcagcgcggctatcgtggctggccacgacgggcgttccttgcgcagctgtgctcgacgttgtcactgaagcgggaagggactggctgctattgggcgaagtgccggggcaggatctcctgtcatctcaccttgctcctgccgagaaagtatccatcatggctgatgcaatgcggcggctgcatacgcttgatccggctacctgcccattcgaccaccaagcgaaacatcgcatcgagcgagcacgtactcggatggaagccggtcttgtcgatcaggatgatctggacgaagagcatcaggggctcgcgccagccgaactgttcgccaggctcaaggcgcgcatgcccgacggcgatgatctcgtcgtgacccatggcgatgcctgcttgccgaatatcatggtggaaaatggccgcttttctggattcatcgactgtggccggctgggtgtggcggaccgctatcaggacatagcgttggctacccgtgatattgctgaagagcttggcggcgaatgggctgaccgcttcctcgtgctttacggtatcgccgctcccgattcgcagcgcatcgccttctatcgccttcttgacgagttcttctgaggggatcaattctctagagctcgctgatcagcctcgactgtgccttctagttgccagccatctgttgtttgcccctcccccgtgccttccttgaccctggaaggtgccactcccactgtcctttcctaataaaatgaggaaattgcatcgcattgtctgagtaggtgtcattctattctggggggtggggtggggcaggacagcaagggggaggattgggaagacaatagcaggcatgctggggatgcggtgggctctatggcttctgaggcggaaagaaccagctggggctcgactagagcttgcggaacccttaatataacttcgtataatgtatgctatacgaagttattaggtccctcgaggggatccactagttctagagcggccgggcaaacatgtgttccctgaacaggaaacagagaa

SEQ ID NO: 20 - DNA, 53 bp, Artificial Sequence
  synthesized_exon 3
gtccctgtcaagaccaaaggcaaacatgtgttccctgaacaggaaacagagaa